European Patent Application EP 4 293 114 A1, published December 20, 2023. Title: Method of preparing nucleic acids sample from skin keratinocytes. Applicant: Kao Corporation. The sequence listing filed with the application follows.

SEQUENCE LISTING (1 sequence)

SEQ ID NO: 1 - protein, 301 aa, Bacteriophage T4
MFKRKSTAELAAQMAKLNGNKGFSSEDKGEWKLKLDNAGNGQAVIRFLPSKNDEQAPFAILVNHGFKKNGKWYIETCSSTHGDYDSCPVCQYISKNDLYNTDNKEYSLVKRKTSYWANILVVKDPAAPENEGKVFKYRFGKKIWDKINAMIAVDVEMGETPVDVTCPWEGANFVLKVKQVSGFSNYDESKFLNQSAIPNIDDESFQKELFEQMVDLSEMTSKDKFKSFEELNTKFGQVMGTAVMGGAAATAAKKADKVADDLDAFNVDDFNTKTEDDFMSSSSGSSSSADDTDLDDLLNDL